European Patent Application EP 4 368 630 A1, published May 15, 2024. Title: Novel antigenic peptide for production of formyl. Applicant: POSTECH Research and Business Development Foundation. The sequence listing filed with the application follows.

SEQUENCE LISTING (1 sequence)

SEQ ID NO: 1 - protein, 5 aa, Artificial
  antigenic protein
  FORMYLATION (1)..(1)
  misc_feature (5)..(5): Xaa can be any naturally occurring amino acid
MGSGX